European Patent Specification EP 4 440 599 B1, published February 25, 2026. Title: Combination of an immunocytokine comprising IL-12 and a kinase inhibitor. Applicant: Philogen, S.P.A. The sequence listing filed with the application follows.

SEQUENCE LISTING (27 sequences)

SEQ ID NO: 1 - protein, 306 aa, synthetic construct
  REGION 1..306: note = immunocytokine sequence
IWELKKDVYVVELDWYPDAPGEMVVLTCDTPEEDGITWTLDQSSEVLGSGKTLTIQVKEFGDAGQYTCHKGGEVLSHSLLLLHKKEDGIWSTDILKDQKEPKNKTFLRCEAKNYSGRFTCWWLTTISTDLTFSVKSSRGSSDPQGVTCGAATLSAERVRGDNKEYEYSVECQEDSACPAAEESLPIEVMVDAVHKLKYENYTSSFFIRDIIKPDPPKNLQLKPLKNSRQVEVSWEYPDTWSTPHSYFSLTFCVQVQGKSKREKKDRVFTDKTSATVICRKNASISVRAQDRYYSSSWSEWASVPCS

SEQ ID NO: 2 - protein, 15 aa, synthetic construct
  REGION 1..15: note = immunocytokine sequence
GGGGSGGGGSGGGGS

SEQ ID NO: 3 - protein, 197 aa, synthetic construct
  REGION 1..197: note = immunocytokine sequence
RNLPVATPDPGMFPCLHHSQNLLRAVSNMLQKARQTLEFYPCTSEEIDHEDITKDKTSTVEACLPLELTKNESCLNSRETSFITNGSCLASRKTSFMMALCLSSIYEDLKMYQVEFKTMNAKLLMDPKRQIFLDQNMLAVIDELMQALNFNSETVPQKSSLEEPDFYKTKIKLCILLHAFRIRAVTIDRVMSYLNAS

SEQ ID NO: 4 - protein, 15 aa, synthetic construct
  REGION 1..15: note = immunocytokine sequence
GSADGGSSAGGSDAG

SEQ ID NO: 5 - protein, 108 aa, synthetic construct [sequence omitted]

SEQ ID NO: 6 - protein, 5 aa, synthetic construct
  REGION 1..5: note = immunocytokine sequence
GSSGG

SEQ ID NO: 7 - protein, 116 aa, synthetic construct [sequence omitted]

SEQ ID NO: 8 - protein, 15 aa, synthetic construct
  REGION 1..15: note = immunocytokine sequence
SSSSGSSSSGSSSSG

SEQ ID NO: 9 - protein, 1006 aa, synthetic construct
  REGION 1..1006: note = immunocytokine sequence
IWELKKDVYVVELDWYPDAPGEMVVLTCDTPEEDGITWTLDQSSEVLGSGKTLTIQVKEFGDAGQYTCHKGGEVLSHSLLLLHKKEDGIWSTDILKDQKEPKNKTFLRCEAKNYSGRFTCWWLTTISTDLTFSVKSSRGSSDPQGVTCGAATLSAERVRGDNKEYEYSVECQEDSACPAAEESLPIEVMVDAVHKLKYENYTSSFFIRDIIKPDPPKNLQLKPLKNSRQVEVSWEYPDTWSTPHSYFSLTFCVQVQGKSKREKKDRVFTDKTSATVICRKNASISVRAQDRYYSSSWSEWASVPCSGGGGSGGGGSGGGGSRNLPVATPDPGMFPCLHHSQNLLRAVSNMLQKARQTLEFYPCTSEEIDHEDITKDKTSTVEACLPLELTKNESCLNSRETSFITNGSCLASRKTSFMMALCLSSIYEDLKMYQVEFKTMNAKLLMDPKRQIFLDQNMLAVIDELMQALNFNSETVPQKSSLEEPDFYKTKIKLCILLHAFRIRAVTIDRVMSYLNASGSADGGSSAGGSDAGEVQLLESGGGLVQPGGSLRLSCAASGFTFSSFSMSWVRQAPGKGLEWVSSISGSSGTTYYADSVKGRFTISRDNSKNTLYLQMNSLRAEDTAVYYCAKPFPYFDYWGQGTLVTVSSGSSGGEIVLTQSPGTLSLSPGERATLSCRASQSVSSSFLAWYQQKPGQAPRLLIYYASSRATGIPDRFSGSGSGTDFTLTISRLEPEDFAVYYCQQTGRIPPTFGQGTKVEIKSSSSGSSSSGSSSSGEVQLLESGGGLVQPGGSLRLSCAASGFTFSSFSMSWVRQAPGKGLEWVSSISGSSGTTYYADSVKGRFTISRDNSKNTLYLQMNSLRAEDTAVYYCAKPFPYFDYWGQGTLVTVSSGSSGGEIVLTQSPGTLSLSPGERATLSCRASQSVSSSFLAWYQQKPGQAPRLLIYYASSRATGIPDRFSGSGSGTDFTLTISRLEPEDFAVYYCQQTGRIPPTFGQGTKVEIK

SEQ ID NO: 10 - protein, 5 aa, synthetic construct
  REGION 1..5: note = immunocytokine sequence
SFSMS

SEQ ID NO: 11 - protein, 17 aa, synthetic construct
  REGION 1..17: note = immunocytokine sequence
SISGSSGTTYYADSVKG

SEQ ID NO: 12 - protein, 7 aa, synthetic construct
  REGION 1..7: note = immunocytokine sequence
PFPYFDY

SEQ ID NO: 13 - protein, 12 aa, synthetic construct
  REGION 1..12: note = immunocytokine sequence
RASQSVSSSFLA

SEQ ID NO: 14 - protein, 7 aa, synthetic construct
  REGION 1..7: note = immunocytokine sequence
YASSRAT

SEQ ID NO: 15 - protein, 9 aa, synthetic construct
  REGION 1..9: note = immunocytokine sequence
QQTGRIPPT

SEQ ID NO: 16 - protein, 313 aa, synthetic construct
  REGION 1..313: note = immunocytokine sequence
MWELEKDVYVVEVDWTPDAPGETVNLTCDTPEEDDITWTSDQRHGVIGSGKTLTITVKEFLDAGQYTCHKGGETLSHSHLLLHKKENGIWSTEILKNFKNKTFLKCEAPNYSGRFTCSWLVQRNMDLKFNIKSSSSSPDSRAVTCGMASLSAEKVTLDQRDYEKYSVSCQEDVTCPTAEETLPIELALEARQQNKYENYSTSFFIRDIIKPDPPKNLQMRPLKNSQVEVSWEYPDSWSTPHSYFSLKFFVRIQRKKEKMKETEEGCNQKGAFLVERTSTEVQCKGGNVCVQAQDRYYNSSCSKWACVPCRVRS

SEQ ID NO: 17 - protein, 193 aa, synthetic construct
  REGION 1..193: note = immunocytokine sequence
RVIPVSGPARCLSQSRNLLKTTDDMVKTAREKLKHYSCTAEDIDHEDITRDQTSTLKTCLPLELHKNESCLATRETSSTTRGSCLPPQKTSLMMTLCLGSIYEDLKMYQTEFQAINAALQNHNHQQIILDKGMLVAIDELMQSLNHNGETLRQKPPVGEADPYRVKMKLCILLHAFSTRVVTINRVMGYLSSA

SEQ ID NO: 18 - protein, 5 aa, synthetic construct
  REGION 1..5: note = immunocytokine sequence
GSADG

SEQ ID NO: 19 - protein, 999 aa, synthetic construct
  REGION 1..999: note = immunocytokine sequence
MWELEKDVYVVEVDWTPDAPGETVNLTCDTPEEDDITWTSDQRHGVIGSGKTLTITVKEFLDAGQYTCHKGGETLSHSHLLLHKKENGIWSTEILKNFKNKTFLKCEAPNYSGRFTCSWLVQRNMDLKFNIKSSSSSPDSRAVTCGMASLSAEKVTLDQRDYEKYSVSCQEDVTCPTAEETLPIELALEARQQNKYENYSTSFFIRDIIKPDPPKNLQMRPLKNSQVEVSWEYPDSWSTPHSYFSLKFFVRIQRKKEKMKETEEGCNQKGAFLVERTSTEVQCKGGNVCVQAQDRYYNSSCSKWACVPCRVRSGGGGSGGGGSGGGGSRVIPVSGPARCLSQSRNLLKTTDDMVKTAREKLKHYSCTAEDIDHEDITRDQTSTLKTCLPLELHKNESCLATRETSSTTRGSCLPPQKTSLMMTLCLGSIYEDLKMYQTEFQAINAALQNHNHQQIILDKGMLVAIDELMQSLNHNGETLRQKPPVGEADPYRVKMKLCILLHAFSTRVVTINRVMGYLSSAGSADGEVQLLESGGGLVQPGGSLRLSCAASGFTFSSFSMSWVRQAPGKGLEWVSSISGSSGTTYYADSVKGRFTISRDNSKNTLYLQMNSLRAEDTAVYYCAKPFPYFDYWGQGTLVTVSSGSSGGEIVLTQSPGTLSLSPGERATLSCRASQSVSSSFLAWYQQKPGQAPRLLIYYASSRATGIPDRFSGSGSGTDFTLTISRLEPEDFAVYYCQQTGRIPPTFGQGTKVEIKSSSSGSSSSGSSSSGEVQLLESGGGLVQPGGSLRLSCAASGFTFSSFSMSWVRQAPGKGLEWVSSISGSSGTTYYADSVKGRFTISRDNSKNTLYLQMNSLRAEDTAVYYCAKPFPYFDYWGQGTLVTVSSGSSGGEIVLTQSPGTLSLSPGERATLSCRASQSVSSSFLAWYQQKPGQAPRLLIYYASSRATGIPDRFSGSGSGTDFTLTISRLEPEDFAVYYCQQTGRIPPTFGQGTKVEIK

SEQ ID NO: 20 - protein, 229 aa, synthetic construct
  REGION 1..229: note = immunocytokine sequence
EVQLLESGGGLVQPGGSLRLSCAASGFTFSSFSMSWVRQAPGKGLEWVSSISGSSGTTYYADSVKGRFTISRDNSKNTLYLQMNSLRAEDTAVYYCAKPFPYFDYWGQGTLVTVSSGSSGGEIVLTQSPGTLSLSPGERATLSCRASQSVSSSFLAWYQQKPGQAPRLLIYYASSRATGIPDRFSGSGSGTDFTLTISRLEPEDFAVYYCQQTGRIPPTFGQGTKVEIK

SEQ ID NO: 21 - protein, 15 aa, synthetic construct
  REGION 1..15: note = immunocytokine sequence
GGGSGGGGSSGGGGS

SEQ ID NO: 22 - protein, 15 aa, synthetic construct
  REGION 1..15: note = immunocytokine sequence
GGGAKGGGGKAGGGS

SEQ ID NO: 23 - protein, 15 aa, synthetic construct
  REGION 1..15: note = immunocytokine sequence
GGGGSGGGGEGGGGS

SEQ ID NO: 24 - protein, 15 aa, synthetic construct
  REGION 1..15: note = immunocytokine sequence
GGGGDGGGGDGGGGS

SEQ ID NO: 25 - protein, 14 aa, synthetic construct
  REGION 1..14: note = immunocytokine sequence
APAPAPAPAPAPAP

SEQ ID NO: 26 - protein, 12 aa, synthetic construct
  REGION 1..12: note = immunocytokine sequence
APAPAPAPAPAP

SEQ ID NO: 27 - protein, 17 aa, synthetic construct
  REGION 1..17: note = immunocytokine sequence
AEAAAKEAAAKEAAAKA